European Patent Application EP 4 682 163 A2, published January 21, 2026. Title: METHOD OF REDUCING CST FLUCTUATION IN NEOVASCULAR AMD BY A RECOMBINANT ADENO-ASSOCIATED VIRUS. Applicant: Adverum Biotechnologies, Inc. The sequence listing filed with the application follows.

SEQUENCE LISTING (41 sequences)

SEQ ID NO: 1 - protein, 10 aa, synthetic construct
LALGETTRPA

SEQ ID NO: 2 - protein, 10 aa, synthetic construct
LANETITRPA

SEQ ID NO: 3 - protein, 10 aa, synthetic construct
LAKAGQANNA

SEQ ID NO: 4 - protein, 10 aa, synthetic construct
LAKDPKTTNA

SEQ ID NO: 5 - protein, 7 aa, synthetic construct
KDTDTTR

SEQ ID NO: 6 - protein, 7 aa, synthetic construct
RAGGSVG

SEQ ID NO: 7 - protein, 7 aa, synthetic construct
AVDTTKF

SEQ ID NO: 8 - protein, 7 aa, synthetic construct
STGKVPN

SEQ ID NO: 9 - protein, 10 aa, synthetic construct
LAKDTDTTRA

SEQ ID NO: 10 - protein, 10 aa, synthetic construct
LARAGGSVGA

SEQ ID NO: 11 - protein, 10 aa, synthetic construct
LAAVDTTKFA

SEQ ID NO: 12 - protein, 10 aa, synthetic construct
LASTGKVPNA

SEQ ID NO: 13 - protein, 735 aa, synthetic construct [sequence omitted]

SEQ ID NO: 14 - protein, 7 aa, synthetic construct
LGETTRP

SEQ ID NO: 15 - protein, 7 aa, synthetic construct
NETITRP

SEQ ID NO: 16 - protein, 7 aa, synthetic construct
KAGQANN

SEQ ID NO: 17 - protein, 7 aa, synthetic construct
KDPKTTN

SEQ ID NO: 18 - protein, 7 aa, synthetic construct
KDTDTTR

SEQ ID NO: 19 - protein, 7 aa, synthetic construct
RAGGSVG

SEQ ID NO: 20 - protein, 7 aa, synthetic construct
AVDTTKF

SEQ ID NO: 21 - protein, 7 aa, synthetic construct
STGKVPN

SEQ ID NO: 22 - DNA, 293 bp, synthetic construct
  source 1..293: mol_type = other DNA
acttacggtaaatggcccgcctggctgaccgcccaacgacccccgcccattgacgtcaataatgacgtatgttcccatagtaacgccaatagggactttccattgacgtcaatgggtggagtatttacggtaaactgcccacttggcagtacatcaagtgtatcatatgccaagtccgccccctattgacgtcaatgacggtaaatggcccgcctggcattatgcccagtacatgaccttacgggactttcctacttggcagtacatctacgtattagtcatcgctattacca

SEQ ID NO: 23 - DNA, 220 bp, synthetic construct
  source 1..220: mol_type = other DNA
tgctgatgcggttttggcagtacaccaatgggcgtggatagcggtttgactcacggggatttccaagtctccaccccattgacgtcaatgggagtttgttttggcaccaaaatcaacgggactttccaaaatgtcgtaataaccccgccccgttgacgcaaatgggcggtaggcgtgtacggtgggaggtctatataagcagagctcgtttagtgaaccg

SEQ ID NO: 24 - DNA, 318 bp, synthetic construct
  source 1..318: mol_type = other DNA
ctcactctcttccgcatcgctgtctgcgagggccagctgttgggctcgcggttgaggacaaactcttcgcggtctttccagtactcttggatcggaaacccgtcggcctccgaacggtactccgccaccgagggacctgagcgagtccgcatcgaccggatcggaaaacctctcgagaaaggcgtctaaccagtcacagtcgcaaggtaggctgagcaccgtggcgggcggcagcgggtggcggtcggggttgtttctggcggaggtgctgctgatgatgtaattaaagtaggcggtcttgagacggcggatggtcga

SEQ ID NO: 25 - DNA, 102 bp, synthetic construct
  source 1..102: mol_type = other DNA
ccagctgttggggtgagtactccctctcaaaagcgggcattacttctgcgctaagattgtcagtttccaaaaacgaggaggatttgatattcacctggcccg

SEQ ID NO: 26 - DNA, 810 bp, synthetic construct
  source 1..810: mol_type = other DNA
ctgttctcatcacatcatatcaaggttatataccatcaatattgccacagatgttacttagccttttaatatttctctaatttagtgtatatgcaatgatagttctctgatttctgagattgagtttctcatgtgtaatgattatttagagtttctctttcatctgttcaaatttttgtctagttttattttttactgatttgtaagacttctttttataatctgcatattacaattctctttactggggtgttgcaaatattttctgtcattctatggcctgacttttcttaatggttttttaattttaaaaataagtcttaatattcatgcaatctaattaacaatcttttctttgtggttaggactttgagtcataagaaatttttctctacactgaagtcatgatggcatgcttctatattattttctaaaagatttaaagttttgccttctccatttagacttataattcactggaatttttttgtgtgtatggtatgacatatgggttcccttttattttttacatataaatatatttccctgtttttctaaaaaagaaaaagatcatcattttcccattgtaaaatgccatatttttttcataggtcacttacatatatcaatgggtctgtttctgagctctactctattttatcagcctcactgtctatccccacacatctcatgctttgctctaaatcttgatatttagtggaacattctttcccattttgttctacaagaatatttttgttattgtctttgggctttctatatacattttgaaatgaggttgacaagtta

SEQ ID NO: 27 - DNA, 202 bp, synthetic construct
  source 1..202: mol_type = other DNA
ctgcccgggtggcatccctgtgacccctccccagtgcctctcctggccctggaagttgccactccagtgcccaccagccttgtcctaataaaattaagttgcatcattttgtctgactaggtgtccttctataatattatggggtggaggggggtggtatggagcaaggggcccaagttgggaagaaacctgtagggcctgc

SEQ ID NO: 28 - DNA, 68 bp, synthetic construct
  source 1..68: mol_type = other DNA
aggcggtcttgagacggcggatggtcgaggtgaggtgtggcaggcttgagatccagctgttggggtga

SEQ ID NO: 29 - DNA, 129 bp, synthetic construct
  source 1..129: mol_type = other DNA
cgctgttttgacctccatagtggacaccgggaccgatccagcctccgcgtctcaggggagatctcgtttagtgaaccgtcagatcctcactctcttccgcatcgctgtctgcgagggccagctgttggg

SEQ ID NO: 30 - DNA, 36 bp, synthetic construct
  source 1..36: mol_type = other DNA
ttgatattcacctggcccgatctggccatacacttg

SEQ ID NO: 31 - DNA, 22 bp, synthetic construct
  source 1..22: mol_type = other DNA
cccaggtccaagtttaaacgcc

SEQ ID NO: 32 - DNA, 77 bp, synthetic construct
  source 1..77: mol_type = other DNA
tctttgggctttctatatacattttgaaatgaggttgacaagttacctaggaaaactgtcttcctgcccgggtggca

SEQ ID NO: 33 - DNA, 1172 bp, synthetic construct
  source 1..1172: mol_type = other DNA
ctctggagacgacttacggtaaatggcccgcctggctgaccgcccaacgacccccgcccattgacgtcaataatgacgtatgttcccatagtaacgccaatagggactttccattgacgtcaatgggtggagtatttacggtaaactgcccacttggcagtacatcaagtgtatcatatgccaagtccgccccctattgacgtcaatgacggtaaatggcccgcctggcattatgcccagtacatgaccttacgggactttcctacttggcagtacatctacgtattagtcatcgctattaccatgctgatgcggttttggcagtacaccaatgggcgtggatagcggtttgactcacggggatttccaagtctccaccccattgacgtcaatgggagtttgttttggcaccaaaatcaacgggactttccaaaatgtcgtaataaccccgccccgttgacgcaaatgggcggtaggcgtgtacggtgggaggtctatataagcagagctcgtttagtgaaccgtcagatcgcctggagaggccatccacgctgttttgacctccatagtggacaccgggaccgatccagcctccgcgtctcaggggagatctcgtttagtgaaccgtcagatcctcactctcttccgcatcgctgtctgcgagggccagctgttgggctcgcggttgaggacaaactcttcgcggtctttccagtactcttggatcggaaacccgtcggcctccgaacggtactccgccaccgagggacctgagcgagtccgcatcgaccggatcggaaaacctctcgagaaaggcgtctaaccagtcacagtcgcaaggtaggctgagcaccgtggcgggcggcagcgggtggcggtcggggttgtttctggcggaggtgctgctgatgatgtaattaaagtaggcggtcttgagacggcggatggtcgaggtgaggtgtggcaggcttgagatccagctgttggggtgagtactccctctcaaaagcgggcattacttctgcgctaagattgtcagtttccaaaaacgaggaggatttgatattcacctggcccgatctggccatacacttgagtgacaatgacatccactttgcctttctctccacaggtgtccactcccaggtccaagtttaaacgccgccaccatg

SEQ ID NO: 34 - DNA, 1043 bp, synthetic construct
  source 1..1043: mol_type = other DNA
actgttctcatcacatcatatcaaggttatataccatcaatattgccacagatgttacttagccttttaatatttctctaatttagtgtatatgcaatgatagttctctgatttctgagattgagtttctcatgtgtaatgattatttagagtttctctttcatctgttcaaatttttgtctagttttattttttactgatttgtaagacttctttttataatctgcatattacaattctctttactggggtgttgcaaatattttctgtcattctatggcctgacttttcttaatggttttttaattttaaaaataagtcttaatattcatgcaatctaattaacaatcttttctttgtggttaggactttgagtcataagaaatttttctctacactgaagtcatgatggcatgcttctatattattttctaaaagatttaaagttttgccttctccatttagacttataattcactggaatttttttgtgtgtatggtatgacatatgggttcccttttattttttacatataaatatatttccctgtttttctaaaaaagaaaaagatcatcattttcccattgtaaaatgccatatttttttcataggtcacttacatatatcaatgggtctgtttctgagctctactctattttatcagcctcactgtctatccccacacatctcatgctttgctctaaatcttgatatttagtggaacattctttcccattttgttctacaagaatatttttgttattgtctttgggctttctatatacattttgaaatgaggttgacaagttacctaggaaaactgtcttcctgcccgggtggcatccctgtgacccctccccagtgcctctcctggccctggaagttgccactccagtgcccaccagccttgtcctaataaaattaagttgcatcattttgtctgactaggtgtccttctataatattatggggtggaggggggtggtatggagcaaggggcccaagttgggaagaaacctgtagggcctgcgaagacagtcag

SEQ ID NO: 35 - protein, 431 aa, synthetic construct
SDTGRPFVEMYSEIPEIIHMTEGRELVIPCRVTSPNITVTLKKFPLDTLIPDGKRIIWDSRKGFIISNATYKEIGLLTCEATVNGHLYKTNYLTHRQTNTIIDVVLSPSHGIELSVGEKLVLNCTARTELNVGIDFNWEYPSSKHQHKKLVNRDLKTQSGSEMKKFLSTLTIDGVTRSDQGLYTCAASSGLMTKKNSTFVRVHEKDKTHTCPPCPAPELLGGPSVFLFPPKPKDTLMISRTPEVTCVVVDVSHEDPEVKFNWYVDGVEVHNAKTKPREEQYNSTYRVVSVLTVLHQDWLNGKEYKCKVSNKALPAPIEKTISKAKGQPREPQVYTLPPSRDELTKNQVSLTCLVKGFYPSDIAVEWESNGQPENNYKTTPPVLDSDGSFFLYSKLTVDKSRWQQGNVFSCSVMHEALHNHYTQKSLSLSPG

SEQ ID NO: 36 - DNA, 1377 bp, synthetic construct
  source 1..1377: mol_type = other DNA
atggtcagctactgggacaccggggtcctgctgtgcgcgctgctcagctgtctgcttctcacaggatctagttccggaagtgataccggtagacctttcgtagagatgtacagtgaaatccccgaaattatacacatgactgaaggaagggagctcgtcattccctgccgggttacgtcacctaacatcactgttactttaaaaaagtttccacttgacactttgatccctgatggaaaacgcataatctgggacagtagaaagggcttcatcatatcaaatgcaacgtacaaagaaatagggcttctgacctgtgaagcaacagtcaatgggcatttgtataagacaaactatctcacacatcgacaaaccaatacaatcatagatgtggttctgagtccgtctcatggaattgaactatctgttggagaaaagcttgtcttaaattgtacagcaagaactgaactaaatgtggggattgacttcaactgggaatacccttcttcgaagcatcagcataagaaacttgtaaaccgagacctaaaaacccagtctgggagtgagatgaagaaatttttgagcaccttaactatagatggtgtaacccggagtgaccaaggattgtacacctgtgcagcatccagtgggctgatgaccaagaagaacagcacatttgtcagggtccatgaaaaggacaaaactcacacatgcccaccgtgcccagcacctgaactcctggggggaccgtcagtcttcctcttccccccaaaacccaaggacaccctcatgatctcccggacccctgaggtcacatgcgtggtggtggacgtgagccacgaagaccctgaggtcaagttcaactggtacgtggacggcgtggaggtgcataatgccaagacaaagccgcgggaggagcagtacaacagcacgtaccgtgtggtcagcgtcctcaccgtcctgcaccaggactggctgaatggcaaggagtacaagtgcaaggtctccaacaaagccctcccagcccccatcgagaaaaccatctccaaagccaaagggcagccccgagaaccacaggtgtacaccctgcccccatcccgggatgagctgaccaagaaccaggtcagcctgacctgcctggtcaaaggcttctatcccagcgacatcgccgtggagtgggagagcaatgggcagccggagaacaactacaagaccacgcctcccgtgctggactccgacggctccttcttcctctacagcaagctcaccgtggacaagagcaggtggcagcaggggaacgtcttctcatgctccgtgatgcatgaggctctgcacaaccactacacgcagaagagcctctccctgtctccgggtaaatga

SEQ ID NO: 37 - protein, 745 aa, synthetic construct
MAADGYLPDWLEDTLSEGIRQWWKLKPGPPPPKPAERHKDDSRGLVLPGYKYLGPFNGLDKGEPVNEADAAALEHDKAYDRQLDSGDNPYLKYNHADAEFQERLKEDTSFGGNLGRAVFQAKKRVLEPLGLVEEPVKTAPGKKRPVEHSPVEPDSSSGTGKAGQQPARKRLNFGQTGDADSVPDPQPLGQPPAAPSGLGTNTMATGSGAPMADNNEGADGVGNSSGNWHCDSTWMGDRVITTSTRTWALPTYNNHLYKQISSQSGASNDNHYFGYSTPWGYFDFNRFHCHFSPRDWQRLINNNWGFRPKRLNFKLFNIQVKEVTQNDGTTTIANNLTSTVQVFTDSEYQLPYVLGSAHQGCLPPFPADVFMVPQYGYLTLNNGSQAVGRSSFYCLEYFPSQMLRTGNNFTFSYTFEDVPFHSSYAHSQSLDRLMNPLIDQYLYYLSRTNTPSGTTTQSRLQFSQAGASDIRDQSRNWLPGPCYRQQRVSKTSADNNNSEYSWTGATKYHLNGRDSLVNPGPAMASHKDDEEKFFPQSGVLIFGKQGSEKTNVDIEKVMITDEEEIRTTNPVATEQYGSVSTNLQRGNLALGETTRPARQAATADVNTQGVLPGMVWQDRDVYLQGPIWAKIPHTDGHFHPSPLMGGFGLKHPPPQILIKNTPVPANPSTTFSAAKFASFITQYSTGQVSVEIEWELQKENSKRWNPEIQYTSNYNKSVNVDFTVDTNGVYSEPRPIGTRYLTRNL

SEQ ID NO: 38 - protein, 250 aa, synthetic construct
FSYTFEDVPFHSSYAHSQSLDRLMNPLIDQYLYYLSRTNTPSGTTTQSRLQFSQAGASDIRDQSRNWLPGPCYRQQRVSKTSADNNNSEYSWTGATKYHLNGRDSLVNPGPAMASHKDDEEKFFPQSGVLIFGKQGSEKTNVDIEKVMITDEEEIRTTNPVATEQYGSVSTNLQRGNLALGETTRPARQAATADVNTQGVLPGMVWQDRDVYLQGPIWAKIPHTDGHFHPSPLMGGFGLKHPPPQILIKN

SEQ ID NO: 39 - DNA, 3916 bp, synthetic construct
  source 1..3916: mol_type = other DNA
gcgcgctcgctcgctcactgaggccgcccgggcaaagcccgggcgtcgggcgacctttggtcgcccggcctcagtgagcgagcgagcgcgcagagagggagtggccaactccatcactaggggttccttgtagttaatgattaacccgccatgctacttatctacgtactctggagacgacttacggtaaatggcccgcctggctgaccgcccaacgacccccgcccattgacgtcaataatgacgtatgttcccatagtaacgccaatagggactttccattgacgtcaatgggtggagtatttacggtaaactgcccacttggcagtacatcaagtgtatcatatgccaagtccgccccctattgacgtcaatgacggtaaatggcccgcctggcattatgcccagtacatgaccttacgggactttcctacttggcagtacatctacgtattagtcatcgctattaccatgctgatgcggttttggcagtacaccaatgggcgtggatagcggtttgactcacggggatttccaagtctccaccccattgacgtcaatgggagtttgttttggcaccaaaatcaacgggactttccaaaatgtcgtaataaccccgccccgttgacgcaaatgggcggtaggcgtgtacggtgggaggtctatataagcagagctcgtttagtgaaccgtcagatcgcctggagaggccatccacgctgttttgacctccatagtggacaccgggaccgatccagcctccgcgtctcaggggagatctcgtttagtgaaccgtcagatcctcactctcttccgcatcgctgtctgcgagggccagctgttgggctcgcggttgaggacaaactcttcgcggtctttccagtactcttggatcggaaacccgtcggcctccgaacggtactccgccaccgagggacctgagcgagtccgcatcgaccggatcggaaaacctctcgagaaaggcgtctaaccagtcacagtcgcaaggtaggctgagcaccgtggcgggcggcagcgggtggcggtcggggttgtttctggcggaggtgctgctgatgatgtaattaaagtaggcggtcttgagacggcggatggtcgaggtgaggtgtggcaggcttgagatccagctgttggggtgagtactccctctcaaaagcgggcattacttctgcgctaagattgtcagtttccaaaaacgaggaggatttgatattcacctggcccgatctggccatacacttgagtgacaatgacatccactttgcctttctctccacaggtgtccactcccaggtccaagtttaaacgccgccaccatggtgtcatactgggatactggagtcttgctttgtgccctgctgtcctgcctcctcctgactggctccagctcgggctcagataccggtcgccccttcgtggagatgtactccgagatcccggaaattatccacatgactgaggggcgcgaacttgtgatcccctgccgggtcaccagcccgaacattactgtgactttgaagaagttccccctggacaccctgattccggatgggaagagaattatctgggattcacggaagggattcatcatcagcaacgcgacctacaaggaaattggcctcctcacttgcgaagccactgtgaacggacacttgtacaagaccaactacctgacccaccgccagaccaacaccatcatcgacgtcgtcctgtccccttcgcacgggatcgagctctcggtgggagagaagttggtgcttaactgcaccgcccggacggaactgaatgtgggaatcgacttcaactgggaatacccgtccagcaagcatcagcataagaagctggtgaaccgggacctcaagactcagtccggcagcgaaatgaagaagttcctgtcgaccctcactattgacggagtgaccagatccgaccagggcctctacacttgcgccgcttccagcggactcatgaccaagaagaacagcactttcgtgagggtgcatgagaaggacaagacccacacgtgtccgccgtgcccagccccagagctgctgggaggcccttccgtgttcctgtttccgcccaagccaaaggataccctgatgatctcaaggacccctgaggtcacatgcgtcgtggtggatgtgtcgcacgaggaccctgaagtcaaattcaattggtatgtggacggagtggaagtccacaacgcgaaaaccaagccgagagaagaacagtacaattccacctaccgggtggtgtcggtgctgactgtgctgcaccaggactggctcaacggaaaggagtacaagtgcaaggtgtccaacaaggctctgcccgcacctattgaaaagaccatctccaaggccaagggtcaacctcgcgagcctcaggtgtacactctgcctccaagccgggacgaactgactaagaaccaagtctctctgacctgtttggtgaagggcttctacccgtcagacatcgcagtggagtgggagtcaaacggtcagccggagaacaactacaaaacaaccccccccgtgctggactccgacggctccttcttcctgtactccaagcttaccgtggataagagccgctggcaacagggcaacgtgttttcctgctccgtcatgcacgaagccctgcacaaccattatacccagaagtccctgtcgctgtcccccgggaaatagtgactgttctcatcacatcatatcaaggttatataccatcaatattgccacagatgttacttagccttttaatatttctctaatttagtgtatatgcaatgatagttctctgatttctgagattgagtttctcatgtgtaatgattatttagagtttctctttcatctgttcaaatttttgtctagttttattttttactgatttgtaagacttctttttataatctgcatattacaattctctttactggggtgttgcaaatattttctgtcattctatggcctgacttttcttaatggttttttaattttaaaaataagtcttaatattcatgcaatctaattaacaatcttttctttgtggttaggactttgagtcataagaaatttttctctacactgaagtcatgatggcatgcttctatattattttctaaaagatttaaagttttgccttctccatttagacttataattcactggaatttttttgtgtgtatggtatgacatatgggttcccttttattttttacatataaatatatttccctgtttttctaaaaaagaaaaagatcatcattttcccattgtaaaatgccatatttttttcataggtcacttacatatatcaatgggtctgtttctgagctctactctattttatcagcctcactgtctatccccacacatctcatgctttgctctaaatcttgatatttagtggaacattctttcccattttgttctacaagaatatttttgttattgtctttgggctttctatatacattttgaaatgaggttgacaagttacctaggaaaactgtcttcctgcccgggtggcatccctgtgacccctccccagtgcctctcctggccctggaagttgccactccagtgcccaccagccttgtcctaataaaattaagttgcatcattttgtctgactaggtgtccttctataatattatggggtggaggggggtggtatggagcaaggggcccaagttgggaagaaacctgtagggcctgcgtacgtagataagtagcatggcgggttaatcattaactacaaggaacccctagtgatggagttggccactccctctctgcgcgctcgctcgctcactgaggccgggcgaccaaaggtcgcccgacgcccgggctttgcccgggcggcctcagtgagcgagcgagcgcgc

SEQ ID NO: 40 - DNA, 1377 bp, synthetic construct
  source 1..1377: mol_type = other DNA
atggtgtcatactgggatactggagtcttgctttgtgccctgctgtcctgcctcctcctgactggctccagctcgggctcagataccggtcgccccttcgtggagatgtactccgagatcccggaaattatccacatgactgaggggcgcgaacttgtgatcccctgccgggtcaccagcccgaacattactgtgactttgaagaagttccccctggacaccctgattccggatgggaagagaattatctgggattcacggaagggattcatcatcagcaacgcgacctacaaggaaattggcctcctcacttgcgaagccactgtgaacggacacttgtacaagaccaactacctgacccaccgccagaccaacaccatcatcgacgtcgtcctgtccccttcgcacgggatcgagctctcggtgggagagaagttggtgcttaactgcaccgcccggacggaactgaatgtgggaatcgacttcaactgggaatacccgtccagcaagcatcagcataagaagctggtgaaccgggacctcaagactcagtccggcagcgaaatgaagaagttcctgtcgaccctcactattgacggagtgaccagatccgaccagggcctctacacttgcgccgcttccagcggactcatgaccaagaagaacagcactttcgtgagggtgcatgagaaggacaagacccacacgtgtccgccgtgcccagccccagagctgctgggaggcccttccgtgttcctgtttccgcccaagccaaaggataccctgatgatctcaaggacccctgaggtcacatgcgtcgtggtggatgtgtcgcacgaggaccctgaagtcaaattcaattggtatgtggacggagtggaagtccacaacgcgaaaaccaagccgagagaagaacagtacaattccacctaccgggtggtgtcggtgctgactgtgctgcaccaggactggctcaacggaaaggagtacaagtgcaaggtgtccaacaaggctctgcccgcacctattgaaaagaccatctccaaggccaagggtcaacctcgcgagcctcaggtgtacactctgcctccaagccgggacgaactgactaagaaccaagtctctctgacctgtttggtgaagggcttctacccgtcagacatcgcagtggagtgggagtcaaacggtcagccggagaacaactacaaaacaaccccccccgtgctggactccgacggctccttcttcctgtactccaagcttaccgtggataagagccgctggcaacagggcaacgtgttttcctgctccgtcatgcacgaagccctgcacaaccattatacccagaagtccctgtcgctgtcccccgggaaatag

SEQ ID NO: 41 - protein, 458 aa, synthetic construct
MVSYWDTGVLLCALLSCLLLTGSSSGSDTGRPFVEMYSEIPEIIHMTEGRELVIPCRVTSPNITVTLKKFPLDTLIPDGKRIIWDSRKGFIISNATYKEIGLLTCEATVNGHLYKTNYLTHRQTNTIIDVVLSPSHGIELSVGEKLVLNCTARTELNVGIDFNWEYPSSKHQHKKLVNRDLKTQSGSEMKKFLSTLTIDGVTRSDQGLYTCAASSGLMTKKNSTFVRVHEKDKTHTCPPCPAPELLGGPSVFLFPPKPKDTLMISRTPEVTCVVVDVSHEDPEVKFNWYVDGVEVHNAKTKPREEQYNSTYRVVSVLTVLHQDWLNGKEYKCKVSNKALPAPIEKTISKAKGQPREPQVYTLPPSRDELTKNQVSLTCLVKGFYPSDIAVEWESNGQPENNYKTTPPVLDSDGSFFLYSKLTVDKSRWQQGNVFSCSVMHEALHNHYTQKSLSLSPGK